European Patent Application EP 4 534 650 A2, published April 9, 2025. Title: DIFFERENTIATION OF HUMAN IPS CELLS TO HUMAN ALVEOLAR TYPE II VIA DEFINITIVE ENDODERM. Applicant: Yale University. Application EP. The sequence listing filed with the application follows.

SEQUENCE LISTING (36 sequences)

SEQ ID NO: 1 - DNA, 19 bp, synthetic construct
  misc_feature 1..19: note = Chemically synthesized
  source 1..19: mol_type = other DNA
tccaagccacactccacga

SEQ ID NO: 2 - DNA, 19 bp, synthetic construct
  misc_feature 1..19: note = Chemically synthesized
  source 1..19: mol_type = other DNA
ttcctctggattccttggg

SEQ ID NO: 3 - DNA, 19 bp, synthetic construct
  misc_feature 1..19: note = Chemically synthesized
  source 1..19: mol_type = other DNA
tgggagccgatgacctatg

SEQ ID NO: 4 - DNA, 19 bp, synthetic construct
  misc_feature 1..19: note = Chemically synthesized
  source 1..19: mol_type = other DNA
gcctccttggccatcttgt

SEQ ID NO: 5 - DNA, 19 bp, synthetic construct
  misc_feature 1..19: note = Chemically synthesized
  source 1..19: mol_type = other DNA
ggacgtgagcaagaacatg

SEQ ID NO: 6 - DNA, 19 bp, synthetic construct
  misc_feature 1..19: note = Chemically synthesized
  source 1..19: mol_type = other DNA
tcgctccagctcgtacacc

SEQ ID NO: 7 - DNA, 21 bp, synthetic construct
  misc_feature 1..21: note = Chemically synthesized
  source 1..21: mol_type = other DNA
ccttcttatcgtggtggtggt

SEQ ID NO: 8 - DNA, 22 bp, synthetic construct
  misc_feature 1..22: note = Chemically synthesized
  source 1..22: mol_type = other DNA
tctccgtgtgtttctggctcat

SEQ ID NO: 9 - DNA, 21 bp, synthetic construct
  misc_feature 1..21: note = Chemically synthesized
  source 1..21: mol_type = other DNA
agcttctactctggtgcacaa

SEQ ID NO: 10 - DNA, 18 bp, synthetic construct
  misc_feature 1..18: note = Chemically synthesized
  source 1..18: mol_type = other DNA
ggtggctgggaattgaga

SEQ ID NO: 11 - DNA, 20 bp, synthetic construct
  misc_feature 1..20: note = Chemically synthesized
  source 1..20: mol_type = other DNA
cctcacttcactgcactgta

SEQ ID NO: 12 - DNA, 20 bp, synthetic construct
  misc_feature 1..20: note = Chemically synthesized
  source 1..20: mol_type = other DNA
caggttttctttccctagct

SEQ ID NO: 13 - DNA, 19 bp, synthetic construct
  misc_feature 1..19: note = Chemically synthesized
  source 1..19: mol_type = other DNA
cccagcagacttcacatgt

SEQ ID NO: 14 - DNA, 20 bp, synthetic construct
  misc_feature 1..20: note = Chemically synthesized
  source 1..20: mol_type = other DNA
cctcccatttccctcgtttt

SEQ ID NO: 15 - DNA, 21 bp, synthetic construct
  misc_feature 1..21: note = Chemically synthesized
  source 1..21: mol_type = other DNA
ccaaattctcctgccagtgac

SEQ ID NO: 16 - DNA, 22 bp, synthetic construct
  misc_feature 1..22: note = Chemically synthesized
  source 1..22: mol_type = other DNA
cacgtggtttccaaacaagaaa

SEQ ID NO: 17 - DNA, 20 bp, synthetic construct
  misc_feature 1..20: note = Chemically synthesized
  source 1..20: mol_type = other DNA
ccctggtcacactggctctc

SEQ ID NO: 18 - DNA, 20 bp, synthetic construct
  misc_feature 1..20: note = Chemically synthesized
  source 1..20: mol_type = other DNA
tcataactggagggtgtgtc

SEQ ID NO: 19 - DNA, 19 bp, synthetic construct
  misc_feature 1..19: note = Chemically synthesized
  source 1..19: mol_type = other DNA
caccgcatctggagaacca

SEQ ID NO: 20 - DNA, 21 bp, synthetic construct
  misc_feature 1..21: note = Chemically synthesized
  source 1..21: mol_type = other DNA
gcccatttcctcggtgtagtt

SEQ ID NO: 21 - DNA, 18 bp, synthetic construct
  misc_feature 1..18: note = Chemically synthesized
  source 1..18: mol_type = other DNA
gggagcggtgaagatgga

SEQ ID NO: 22 - DNA, 22 bp, synthetic construct
  misc_feature 1..22: note = Chemically synthesized
  source 1..22: mol_type = other DNA
tcatgttgctcacggaggagta

SEQ ID NO: 23 - DNA, 18 bp, synthetic construct
  misc_feature 1..18: note = Chemically synthesized
  source 1..18: mol_type = other DNA
ggcgcagcagaatccaga

SEQ ID NO: 24 - DNA, 18 bp, synthetic construct
  misc_feature 1..18: note = Chemically synthesized
  source 1..18: mol_type = other DNA
ccacgacttgcccagcat

SEQ ID NO: 25 - DNA, 21 bp, synthetic construct
  misc_feature 1..21: note = Chemically synthesized
  source 1..21: mol_type = other DNA
gttatgttgctggacatgggt

SEQ ID NO: 26 - DNA, 22 bp, synthetic construct
  misc_feature 1..22: note = Chemically synthesized
  source 1..22: mol_type = other DNA
gaagccgtgacagaatgactac

SEQ ID NO: 27 - DNA, 19 bp, synthetic construct
  misc_feature 1..19: note = Chemically synthesized
  source 1..19: mol_type = other DNA
gctcctacgactattgccc

SEQ ID NO: 28 - DNA, 19 bp, synthetic construct
  misc_feature 1..19: note = Chemically synthesized
  source 1..19: mol_type = other DNA
cgtattccttgcttgccct

SEQ ID NO: 29 - DNA, 24 bp, synthetic construct
  misc_feature 1..24: note = Chemically synthesized
  source 1..24: mol_type = other DNA
attgcagtggttatcatcggagtg

SEQ ID NO: 30 - DNA, 24 bp, synthetic construct
  misc_feature 1..24: note = Chemically synthesized
  source 1..24: mol_type = other DNA
ctcgttgttggagttcagaagtgg

SEQ ID NO: 31 - DNA, 20 bp, synthetic construct
  misc_feature 1..20: note = Chemically synthesized
  source 1..20: mol_type = other DNA
tttcttacccaagccactgc

SEQ ID NO: 32 - DNA, 21 bp, synthetic construct
  misc_feature 1..21: note = Chemically synthesized
  source 1..21: mol_type = other DNA
ttctcttcatattcctggtgg

SEQ ID NO: 33 - DNA, 21 bp, synthetic construct
  misc_feature 1..21: note = Chemically synthesized
  source 1..21: mol_type = other DNA
aaacgccagtaagtgacagag

SEQ ID NO: 34 - DNA, 21 bp, synthetic construct
  misc_feature 1..21: note = Chemically synthesized
  source 1..21: mol_type = other DNA
atatctgcatggaaggtgaat

SEQ ID NO: 35 - DNA, 23 bp, synthetic construct
  misc_feature 1..23: note = Chemically synthesized
  source 1..23: mol_type = other DNA
gacaacagcctcaagatcatcag

SEQ ID NO: 36 - DNA, 23 bp, synthetic construct
  misc_feature 1..23: note = Chemically synthesized
  source 1..23: mol_type = other DNA
atggcatggactgtggtcatgag